European Patent Application EP 4 636 090 A1, published October 22, 2025. Title: UTR for improving translation efficiency and/or stability of RNA molecule and use thereof. Applicant: SHENZHEN SHENXIN BIOTECHNOLOGY CO., LTD. The sequence listing filed with the application follows.

SEQUENCE LISTING (56 sequences)

SEQ ID NO: 1 - DNA, 35 bp, synthetic construct
  source 1..35: mol_type = other DNA
actcttctggtccccacagactcagagagaaccca

SEQ ID NO: 2 - DNA, 23 bp, synthetic construct
  source 1..23: mol_type = other DNA
gacggacggggtcaggtcccatc

SEQ ID NO: 3 - DNA, 13 bp, synthetic construct
  source 1..13: mol_type = other DNA
cagctacgacgcc

SEQ ID NO: 4 - DNA, 58 bp, synthetic construct
  source 1..58: mol_type = other DNA
aggcacagacaccaaggacagagacgctggctaggccgccctccccactgttaccaac

SEQ ID NO: 5 - DNA, 62 bp, synthetic construct
  source 1..62: mol_type = other DNA
aggattccaaggcccaactccccgaaccactcagggtcctgtggacagctcacctagctgca

SEQ ID NO: 6 - DNA, 50 bp, synthetic construct
  source 1..50: mol_type = other DNA
acatttgcttctgacacaactgtgttcactagcaacctcaaacagacacc

SEQ ID NO: 7 - DNA, 61 bp, synthetic construct
  source 1..61: mol_type = other DNA
aactctatatagggagttcaactggtcacccagagctgtcctgtggcctctgcagctcagc

SEQ ID NO: 8 - DNA, 78 bp, synthetic construct
  source 1..78: mol_type = other DNA
ctcattgaactcgcctgcagctcttgggttttttgtggcttccttcgttattggagccaggcctacaccccagcaacc

SEQ ID NO: 9 - DNA, 83 bp, synthetic construct
  source 1..83: mol_type = other DNA
gaacgtggtataaaaggggcgggaggccaggctcgtgccgttttgcagacgccaccgccgaggaaaaccgtgtactattagcc

SEQ ID NO: 10 - DNA, 78 bp, synthetic construct
  source 1..78: mol_type = other DNA
gacaactcggtggtggccactgcgcagaccagacttcgctcgtactcgtgcgcctcgcttcgcttttcctccgcaacc

SEQ ID NO: 11 - DNA, 73 bp, synthetic construct
  source 1..73: mol_type = other DNA
atacatagtttactttcatttttgactctgaggctctttccaacgctgtaaaaaaggacagaggctgttccct

SEQ ID NO: 12 - DNA, 84 bp, synthetic construct
  source 1..84: mol_type = other DNA
cggaggctcggccacaacgccactggattggtggtagggcggggcgggccacagtctccagcctgaagcggaagtggaggaaag

SEQ ID NO: 13 - DNA, 67 bp, synthetic construct
  source 1..67: mol_type = other DNA
agaacctagagcccaaggttcagagtcacccatctcagcaagcccagaagtatctgcaatatctacg

SEQ ID NO: 14 - DNA, 44 bp, synthetic construct
  source 1..44: mol_type = other DNA
ccgggcgctcctagcggcctcccggaccctgccgccctgccact

SEQ ID NO: 15 - DNA, 96 bp, synthetic construct
  source 1..96: mol_type = other DNA
agtgcgtctggccggcgctttatagctgcagcctgggcggctccgctagctgtttttcgtcttccctaggctatttctgccgggcgctccgcgaag

SEQ ID NO: 16 - DNA, 32 bp, synthetic construct
  source 1..32: mol_type = other DNA
gccccagcttggccgggcgcggagcggggcgc

SEQ ID NO: 17 - DNA, 29 bp, synthetic construct
  source 1..29: mol_type = other DNA
gagaccccagcggcgggcggtggacagtc

SEQ ID NO: 18 - DNA, 44 bp, synthetic construct
  source 1..44: mol_type = other DNA
cttccatctgcccagagaggagcatctggatcaaggtgctggcc

SEQ ID NO: 19 - DNA, 136 bp, synthetic construct
  source 1..136: mol_type = other DNA
gttgactaagtcaataatcagaatcagcaggtttgcagtcagattggcagggataagcagcctagctcaggagaagtgagtataaaagccccaggctgggagcagccatcacagaagtccactcattcttggcagg

SEQ ID NO: 20 - DNA, 103 bp, synthetic construct
  source 1..103: mol_type = other DNA
gttgtggctgtggagcggaagtgggtctcaaccactataaatcctctctgtgcccgtccggagctggtgaggacagcctgccagagtctggtctctggacact

SEQ ID NO: 21 - DNA, 181 bp, synthetic construct
  source 1..181: mol_type = other DNA
ggaacgccaaccgcctgggcctagcgcagcttcctccgcccaccacggaagtgaggcggggatactaaagcgacggagcccggtggacggaagtgggtgttggaggctttaaggtagctttaaattcgtgttgtcctgggagctcgcccttttcggctggagtcgggctttacggcgccgg

SEQ ID NO: 22 - DNA, 50 bp, synthetic construct
  source 1..50: mol_type = other DNA
accagccttgggaaattacaatgttttacaataaacagaaagccaagcgg

SEQ ID NO: 23 - DNA, 64 bp, synthetic construct
  source 1..64: mol_type = other DNA
tatggaaactaacaaaattgaccttgcatcatcttctgcaatgtagtaaagaaattctatttgc

SEQ ID NO: 24 - DNA, 83 bp, synthetic construct
  source 1..83: mol_type = other DNA
gccttccagggcagggtgggctccagttgtcttgagggtccggatgggctcaggtaataaagaaacggaagcagcagccagcc

SEQ ID NO: 25 - DNA, 55 bp, synthetic construct
  source 1..55: mol_type = other DNA
ggccctgctgatccgcaccccattcctcccctcccatggccaaaaaccccactgt

SEQ ID NO: 26 - DNA, 82 bp, synthetic construct
  source 1..82: mol_type = other DNA
gtgcccctgccactccgagataaccagtggatgcccaggatcttttaccacaacccctctgtaataaaagagatttgacact

SEQ ID NO: 27 - DNA, 77 bp, synthetic construct
  source 1..77: mol_type = other DNA
ctcctgagggggtacaggagaggccgctgctgccagccgtcatataaaactatttattcataaatattttccaaaat

SEQ ID NO: 28 - DNA, 72 bp, synthetic construct
  source 1..72: mol_type = other DNA
ctctcgggaccaagcaaccttctggaaaacgggttaataaataaatcaataaagaaccttcaagtttctact

SEQ ID NO: 29 - DNA, 173 bp, synthetic construct
  source 1..173: mol_type = other DNA
ggggccttctgacatgagtctggcctggccccacctcctagttcctcataataaagacagattgcttcttcgcttctcactgaggggccttctgacatgagtctggcctggccccacctccccagtttctcataataaagacagattgcttcttcacttgaatcaagggacct

SEQ ID NO: 30 - DNA, 294 bp, synthetic construct
  source 1..294: mol_type = other DNA
agagaacactggacaacattttactactgagggaaatagccaaaaaggcaaataatggaaaaatagtaaacattaagtaaatgctgtagaagtgagtttgtaaatattctacacatgtaaaatatgtaaaactatgggttatttttattaaatgtattttaaaataaaaatttaattctggtttttctgattagagtgcaaaagtgagaaaagttcaatactcttgaaatgtagaattgaaaatgcattagggaaaacttaataaaaattattaccagttatttggaagatctg

SEQ ID NO: 31 - DNA, 119 bp, synthetic construct
  source 1..119: mol_type = other DNA
ggacctgaagggtgacatcccaggaggggcctctgaaatttcccacaccccagcgcctgtgctgaggactccctccatgtggccccaggtgccaccaataaaaatcctacagaaaattc

SEQ ID NO: 32 - DNA, 311 bp, synthetic construct
  source 1..311: mol_type = other DNA
cagccagaccccccatcagtggacaaggggagagtcccctactcccctgatcccccaggttcagactgagctcccccttcccagtagctcttgcatcctcctcccaactctagcctgattcttttcaataaaaaatacaattcaagttgcttctcatggatggcactgcttttctgaggactcaagggccaagatggaggggctgactcagtccagccaacatttaatgagcacctactttatgtatggagctctaacccatgggtccatgggaataaagcagtgaatagtaacaataaataatcgtaaca

SEQ ID NO: 33 - DNA, 200 bp, synthetic construct
  source 1..200: mol_type = other DNA
gacccctggaccaccagccccagcaagagcacaagaggaagagagagaccctcactgctggggagtccctgccacactcagtcccccaccacactgaatctcccctcctcacagttgccatgtagaccccttgaagaggggaggggcctagggagccgcaccttgtcatgtaccatcaataaagtaccctgtgctcaacc

SEQ ID NO: 34 - DNA, 242 bp, synthetic construct
  source 1..242: mol_type = other DNA
gccaaccaagtgtagatgtagcattgttccacacatttaaaacatttgaaggacctaaattcgtagcaaattctgtggcagttttaaaaagttaagctgctatagtaagttactgggcattctcaatacttgaatatggaacatatgcacaggggaaggaaataacattgcactttataaacactgtattgtaagtggaaaatgcaatgtcttaaataaaactatttaaaattggcaccata

SEQ ID NO: 35 - DNA, 120 bp, synthetic construct
  source 1..120: mol_type = other DNA
caggacacagccttggatcaggacagagacttgggggccatcctgcccctccaacccgacatgtgtacctcagctttttccctcacttgcatcaataacttctgtgtttggaacagctaa

SEQ ID NO: 36 - DNA, 248 bp, synthetic construct
  source 1..248: mol_type = other DNA
cctcgtctgtcccttccccttcaccgctccccacagctttgcacccctttcctccccatacacacacaaaccattttattttttgggccattaccccataccccttattgctgccaaaaccacatgggctgggggccagggctggatggacagacacctccccctacccatatccctcccgtgtgtggttggaaaacttttgttttttggggttttttttttctgaataaaaaagattctactaacaa

SEQ ID NO: 37 - DNA, 239 bp, synthetic construct
  source 1..239: mol_type = other DNA
caatatcaagaatctagtttcatctgagaacttctgattagctctcagtcttcagctctatttatcttaggagtttaatttgcccttctctccccatcttccctcagttcccataaaaccttcattacacataaagatacacgtgggggtcagtgaatctgcttgcctttcctgaaagtttctggggcttaagattccagactctgattcattaaactatagtcacccgtgtcctgtga

SEQ ID NO: 38 - DNA, 234 bp, synthetic construct
  source 1..234: mol_type = other DNA
cgaaaccccagggacagcaggaccttcgacgctggaaggatagcctcgcttcccaggtgcagctcccggcaggtctggacagttccacagagcacggtactggccctgtcctcagttcccgtccacccttcaaccagtggctcctgggagacttttcctccctgcctcagctccctgcccagccagcctcctgtctccagagaagttctccattaaaaaataatttagcaaatc

SEQ ID NO: 39 - DNA, 289 bp, synthetic construct
  source 1..289: mol_type = other DNA
aagcaggccaggtgcggtggctcacgcctgtaatcccagccctttgggaggccaaggcgggtggatcacttgaggtcaggagttcaagaccagcctggccaacatggtgaaacctcgtctctactaaaaatacaaaaatcaaccaggcatgacggtgcacgcctgttatcacagctacttgggaagcagcggctggagaattgcttgaacctgggaagtcgaggctgcaagtgagctgagatcatgccatggcagtctagcctgggcaacagagcgagactctgtttca

SEQ ID NO: 40 - DNA, 112 bp, synthetic construct
  source 1..112: mol_type = other DNA
agtgtccagaccattgtcttccaaccccagctggcctctagaacacccactggccagtcctagagctcctgtccctacccactctttgctacaataaatgctgaatgaatcc

SEQ ID NO: 41 - DNA, 344 bp, synthetic construct
  source 1..344: mol_type = other DNA
catcacatttaaaagcatctcagcctaccatgagaataagagaaagaaaatgaagatcaacagcttattcatctgtttttctttttcgttggtgtaaagccaacaccctgtctaaaaaacataaatttctttaatcattttgcctcttttctctgtgcttcaattaataaaaaatggaaagaatctaatagagtggtacagcactgttatttttcaaagatgtgttgctatcctgaaaattctgtaggttctgtggaagttccagtgttctctcttattccacttcggtagaggatttctagtttcttgtgggctaattaaataaatcattaatactcttctaa

SEQ ID NO: 42 - DNA, 355 bp, synthetic construct
  source 1..355: mol_type = other DNA
tgctctgtgggagggactttgctgatttcccctcttcccttcaacatgaaaatatatacccccccatgcagtctaaaatgcttcagtacttgtgaaacacagctgttcttctgttctgcagacacgccttcccctcagccacacccaggcacttaagcacaagcagagtgcacagctgtccactgggccattgtggtgtgagcttcagatggtgaagcattctccccagtgtatgtcttgtatccgatatctaacgctttaaatggctactttggtttctgtctgtaagttaagaccttggatgtggtttaattgtttgtcctcaaaaggaataaaacttttctgctgataagat

SEQ ID NO: 43 - DNA, 233 bp, synthetic construct
  source 1..233: mol_type = other DNA
cttctctgataccagctggaggttgagctcttcttaaagtattcttctcttccttttatcagtaggtgcccagaataagttattgcagtttatcattcaagtgtaaaatattttgaatcaataatatattttctgttttcttttggtaaagactggcttttattaatgcactttctatcctctgtaaactttttgtgctgaatgttgggactgctaaataaaatttgttgcat

SEQ ID NO: 44 - DNA, 130 bp, synthetic construct
  source 1..130: mol_type = other DNA
agtaagcaagcaccttaagtagtgtgttaatgattgaaactgtaattgccttcgggttgtgctttagtctgtaaaattctaaaggagagctgctaaattgttttcttaataaacatttttctcatttgta

SEQ ID NO: 45 - DNA, 112 bp, synthetic construct
  source 1..112: mol_type = other DNA
aaatggaagccacaagcagcccagccctccttaatcaacttcaaggagcaccttcattagtacagcttgcatatttaacattttgtatttcaataaaagtgaagacaaacga

SEQ ID NO: 46 - DNA, 147 bp, synthetic construct
  source 1..147: mol_type = other DNA
cctgctgcctgcccccagcccccttcccggaccccctgtacagcgtccccacctatttcaaatcttatttaacaccccacacccacccctcagttgggacaaataaaggattctcatgggaaggggaggacccctccttcccaactt

SEQ ID NO: 47 - DNA, 111 bp, synthetic construct
  source 1..111: mol_type = other DNA
cctgtgcccgggcatggcctggcagctctccagcagggcagagtgtttgcccaccagctgctagccctaggaaggccaggagcccagtagccatgtggccagtctaccatg

SEQ ID NO: 48 - DNA, 158 bp, synthetic construct
  source 1..158: mol_type = other DNA
ttgggcgacttctctcccccgtccccgtggacacgccccacccgctcggtcctggacacactgcccccctctcttgcctccacccctctgcggactctgcagctccgcggccccggcgcagggagagggagggcacgggcgcgggccgggcctcaagg

SEQ ID NO: 49 - DNA, 100 bp, synthetic construct
  source 1..100: mol_type = other DNA
cgggtggcatccctgtgacccctccccagtgcctctcctggccctggaagttgccactccagtgcccaccagccttgtcctaataaaattaagttgcatc

SEQ ID NO: 50 - DNA, 7040 bp, synthetic construct
  source 1..7040: mol_type = other DNA
gacggatcgggagatctcccgatcccctatggtgcactctcagtacaatctgctctgatgccgcatagttaagccagtatctgctccctgcttgtgtgttggaggtcgctgagtagtgcgcgagcaaaatttaagctacaacaaggcaaggcttgaccgacaattgcatgaagaatctgcttagggttaggcgttttgcgctgcttcgcgatgtacgggccagatatacgcgttgacattgattattgactagttattaatagtaatcaattacggggtcattagttcatagcccatatatggagttccgcgttacataacttacggtaaatggcccgcctggctgaccgcccaacgacccccgcccattgacgtcaataatgacgtatgttcccatagtaacgccaatagggactttccattgacgtcaatgggtggagtatttacggtaaactgcccacttggcagtacatcaagtgtatcatatgccaagtacgccccctattgacgtcaatgacggtaaatggcccgcctggcattatgcccagtacatgaccttatgggactttcctacttggcagtacatctacgtattagtcatcgctattaccatggtgatgcggttttggcagtacatcaatgggcgtggatagcggtttgactcacggggatttccaagtctccaccccattgacgtcaatgggagtttgttttggcaccaaaatcaacgggactttccaaaatgtcgtaacaactccgccccattgacgcaaatgggcggtaggcgtgtacggtgggaggtctatataagcagagctctctggctaactagagaacccactgcttactggcttatcgaaattaatacgactcactatagggagacccaagcttggcattccggtactgttggtaaagccaccatggaagacgccaaaaacataaagaaaggcccggcgccattctatccgctggaagatggaaccgctggagagcaactgcataaggctatgaagagatacgccctggttcctggaacaattgcttttacagatgcacatatcgaggtggacatcacttacgctgagtacttcgaaatgtccgttcggttggcagaagctatgaaacgatatgggctgaatacaaatcacagaatcgtcgtatgcagtgaaaactctcttcaattctttatgccggtgttgggcgcgttatttatcggagttgcagttgcgcccgcgaacgacatttataatgaacgtgaattgctcaacagtatgggcatttcgcagcctaccgtggtgttcgtttccaaaaaggggttgcaaaaaattttgaacgtgcaaaaaaagctcccaatcatccaaaaaattattatcatggattctaaaacggattaccagggatttcagtcgatgtacacgttcgtcacatctcatctacctcccggttttaatgaatacgattttgtgccagagtccttcgatagggacaagacaattgcactgatcatgaactcctctggatctactggtctgcctaaaggtgtcgctctgcctcatagaactgcctgcgtgagattctcgcatgccagagatcctatttttggcaatcaaatcattccggatactgcgattttaagtgttgttccattccatcacggttttggaatgtttactacactcggatatttgatatgtggatttcgagtcgtcttaatgtatagatttgaagaagagctgtttctgaggagccttcaggattacaagattcaaagtgcgctgctggtgccaaccctattctccttcttcgccaaaagcactctgattgacaaatacgatttatctaatttacacgaaattgcttctggtggcgctcccctctctaaggaagtcggggaagcggttgccaagaggttccatctgccaggtatcaggcaaggatatgggctcactgagactacatcagctattctgattacacccgagggggatgataaaccgggcgcggtcggtaaagttgttccattttttgaagcgaaggttgtggatctggataccgggaaaacgctgggcgttaatcaaagaggcgaactgtgtgtgagaggtcctatgattatgtccggttatgtaaacaatccggaagcgaccaacgccttgattgacaaggatggatggctacattctggagacatagcttactgggacgaagacgaacacttcttcatcgttgaccgcctgaagtctctgattaagtacaaaggctatcaggtggctcccgctgaattggaatccatcttgctccaacaccccaacatcttcgacgcaggtgtcgcaggtcttcccgacgatgacgccggtgaacttcccgccgccgttgttgttttggagcacggaaagacgatgacggaaaaagagatcgtggattacgtcgccagtcaagtaacaaccgcgaaaaagttgcgcggaggagttgtgtttgtggacgaagtaccgaaaggtcttaccggaaaactcgacgcaagaaaaatcagagagatcctcataaaggccaagaagggcggaaagatcgccgtgtaattctagagggccctattctatagtgtcacctaaatgctagagctcgctgatcagcctcgactgtgccttctagttgccagccatctgttgtttgcccctcccccgtgccttccttgaccctggaaggtgccactcccactgtcctttcctaataaaatgaggaaattgcatcgcattgtctgagtaggtgtcattctattctggggggtggggtggggcaggacagcaagggggaggattgggaagacaatagcaggcatgctggggatgcggtgggctctatggcttctgaggcggaaagaaccagctggggctctagggggtatccccacgcgccctgtagcggcgcattaagcgcggcgggtgtggtggttacgcgcagcgtgaccgctacacttgccagcgccctagcgcccgctcctttcgctttcttcccttcctttctcgccacgttcgccggctttccccgtcaagctctaaatcgggggctccctttagggttccgatttagtgctttacggcacctcgaccccaaaaaacttgattagggtgatggttcacgtagtgggccatcgccctgatagacggtttttcgccctttgacgttggagtccacgttctttaatagtggactcttgttccaaactggaacaacactcaaccctatctcggtctattcttttgatttataagggattttgccgatttcggcctattggttaaaaaatgagctgatttaacaaaaatttaacgcgaattaattctgtggaatgtgtgtcagttagggtgtggaaagtccccaggctccccagcaggcagaagtatgcaaagcatgcatctcaattagtcagcaaccaggtgtggaaagtccccaggctccccagcaggcagaagtatgcaaagcatgcatctcaattagtcagcaaccatagtcccgcccctaactccgcccatcccgcccctaactccgcccagttccgcccattctccgccccatggctgactaattttttttatttatgcagaggccgaggccgcctctgcctctgagctattccagaagtagtgaggaggcttttttggaggcctaggcttttgcaaaaagctcccgggagcttgtatatccattttcggatctgatcaagagacaggatgaggatcgtttcgcatgattgaacaagatggattgcacgcaggttctccggccgcttgggtggagaggctattcggctatgactgggcacaacagacaatcggctgctctgatgccgccgtgttccggctgtcagcgcaggggcgcccggttctttttgtcaagaccgacctgtccggtgccctgaatgaactgcaggacgaggcagcgcggctatcgtggctggccacgacgggcgttccttgcgcagctgtgctcgacgttgtcactgaagcgggaagggactggctgctattgggcgaagtgccggggcaggatctcctgtcatctcaccttgctcctgccgagaaagtatccatcatggctgatgcaatgcggcggctgcatacgcttgatccggctacctgcccattcgaccaccaagcgaaacatcgcatcgagcgagcacgtactcggatggaagccggtcttgtcgatcaggatgatctggacgaagagcatcaggggctcgcgccagccgaactgttcgccaggctcaaggcgcgcatgcccgacggcgaggatctcgtcgtgacccatggcgatgcctgcttgccgaatatcatggtggaaaatggccgcttttctggattcatcgactgtggccggctgggtgtggcggaccgctatcaggacatagcgttggctacccgtgatattgctgaagagcttggcggcgaatgggctgaccgcttcctcgtgctttacggtatcgccgctcccgattcgcagcgcatcgccttctatcgccttcttgacgagttcttctgagcgggactctggggttcgaaatgaccgaccaagcgacgcccaacctgccatcacgagatttcgattccaccgccgccttctatgaaaggttgggcttcggaatcgttttccgggacgccggctggatgatcctccagcgcggggatctcatgctggagttcttcgcccaccccaacttgtttattgcagcttataatggttacaaataaagcaatagcatcacaaatttcacaaataaagcatttttttcactgcattctagttgtggtttgtccaaactcatcaatgtatcttatcatgtctgtataccgtcgacctctagctagagcttggcgtaatcatggtcatagctgtttcctgtgtgaaattgttatccgctcacaattccacacaacatacgagccggaagcataaagtgtaaagcctggggtgcctaatgagtgagctaactcacattaattgcgttgcgctcactgcccgctttccagtcgggaaacctgtcgtgccagctgcattaatgaatcggccaacgcgcggggagaggcggtttgcgtattgggcgctcttccgcttcctcgctcactgactcgctgcgctcggtcgttcggctgcggcgagcggtatcagctcactcaaaggcggtaatacggttatccacagaatcaggggataacgcaggaaagaacatgtgagcaaaaggccagcaaaaggccaggaaccgtaaaaaggccgcgttgctggcgtttttccataggctccgcccccctgacgagcatcacaaaaatcgacgctcaagtcagaggtggcgaaacccgacaggactataaagataccaggcgtttccccctggaagctccctcgtgcgctctcctgttccgaccctgccgcttaccggatacctgtccgcctttctcccttcgggaagcgtggcgctttctcatagctcacgctgtaggtatctcagttcggtgtaggtcgttcgctccaagctgggctgtgtgcacgaaccccccgttcagcccgaccgctgcgccttatccggtaactatcgtcttgagtccaacccggtaagacacgacttatcgccactggcagcagccactggtaacaggattagcagagcgaggtatgtaggcggtgctacagagttcttgaagtggtggcctaactacggctacactagaagaacagtatttggtatctgcgctctgctgaagccagttaccttcggaaaaagagttggtagctcttgatccggcaaacaaaccaccgctggtagcggtggtttttttgtttgcaagcagcagattacgcgcagaaaaaaaggatctcaagaagatcctttgatcttttctacggggtctgacgctcagtggaacgaaaactcacgttaagggattttggtcatgagattatcaaaaaggatcttcacctagatccttttaaattaaaaatgaagttttaaatcaatctaaagtatatatgagtaaacttggtctgacagttaccaatgcttaatcagtgaggcacctatctcagcgatctgtctatttcgttcatccatagttgcctgactccccgtcgtgtagataactacgatacgggagggcttaccatctggccccagtgctgcaatgataccgcgagacccacgctcaccggctccagatttatcagcaataaaccagccagccggaagggccgagcgcagaagtggtcctgcaactttatccgcctccatccagtctattaattgttgccgggaagctagagtaagtagttcgccagttaatagtttgcgcaacgttgttgccattgctacaggcatcgtggtgtcacgctcgtcgtttggtatggcttcattcagctccggttcccaacgatcaaggcgagttacatgatcccccatgttgtgcaaaaaagcggttagctccttcggtcctccgatcgttgtcagaagtaagttggccgcagtgttatcactcatggttatggcagcactgcataattctcttactgtcatgccatccgtaagatgcttttctgtgactggtgagtactcaaccaagtcattctgagaatagtgtatgcggcgaccgagttgctcttgcccggcgtcaatacgggataataccgcgccacatagcagaactttaaaagtgctcatcattggaaaacgttcttcggggcgaaaactctcaaggatcttaccgctgttgagatccagttcgatgtaacccactcgtgcacccaactgatcttcagcatcttttactttcaccagcgtttctgggtgagcaaaaacaggaaggcaaaatgccgcaaaaaagggaataagggcgacacggaaatgttgaatactcatactcttcctttttcaatattattgaagcatttatcagggttattgtctcatgagcggatacatatttgaatgtatttagaaaaataaacaaataggggttccgcgcacatttccccgaaaagtgccacctgacgtc

SEQ ID NO: 51 - DNA, 7041 bp, synthetic construct
  source 1..7041: mol_type = other DNA
gacggatcgggagatctcccgatcccctatggtgcactctcagtacaatctgctctgatgccgcatagttaagccagtatctgctccctgcttgtgtgttggaggtcgctgagtagtgcgcgagcaaaatttaagctacaacaaggcaaggcttgaccgacaattgcatgaagaatctgcttagggttaggcgttttgcgctgcttcgcgatgtacgggccagatatacgcgttgacattgattattgactagttattaatagtaatcaattacggggtcattagttcatagcccatatatggagttccgcgttacataacttacggtaaatggcccgcctggctgaccgcccaacgacccccgcccattgacgtcaataatgacgtatgttcccatagtaacgccaatagggactttccattgacgtcaatgggtggagtatttacggtaaactgcccacttggcagtacatcaagtgtatcatatgccaagtacgccccctattgacgtcaatgacggtaaatggcccgcctggcattatgcccagtacatgaccttatgggactttcctacttggcagtacatctacgtattagtcatcgctattaccatggtgatgcggttttggcagtacatcaatgggcgtggatagcggtttgactcacggggatttccaagtctccaccccattgacgtcaatgggagtttgttttggcaccaaaatcaacgggactttccaaaatgtcgtaacaactccgccccattgacgcaaatgggcggtaggcgtgtacggtgggaggtctatataagcagagctctctggctaactagagaacccactgcttactggcttatcgaaattaatacgactcactatagggaaagcttgatcagaacggatccgccaccatggaagacgccaaaaacataaagaaaggcccggcgccattctatccgctggaagatggaaccgctggagagcaactgcataaggctatgaagagatacgccctggttcctggaacaattgcttttacagatgcacatatcgaggtggacatcacttacgctgagtacttcgaaatgtccgttcggttggcagaagctatgaaacgatatgggctgaatacaaatcacagaatcgtcgtatgcagtgaaaactctcttcaattctttatgccggtgttgggcgcgttatttatcggagttgcagttgcgcccgcgaacgacatttataatgaacgtgaattgctcaacagtatgggcatttcgcagcctaccgtggtgttcgtttccaaaaaggggttgcaaaaaattttgaacgtgcaaaaaaagctcccaatcatccaaaaaattattatcatggattctaaaacggattaccagggatttcagtcgatgtacacgttcgtcacatctcatctacctcccggttttaatgaatacgattttgtgccagagtccttcgatagggacaagacaattgcactgatcatgaactcctctggatctactggtctgcctaaaggtgtcgctctgcctcatagaactgcctgcgtgagattctcgcatgccagagatcctatttttggcaatcaaatcattccggatactgcgattttaagtgttgttccattccatcacggttttggaatgtttactacactcggatatttgatatgtggatttcgagtcgtcttaatgtatagatttgaagaagagctgtttctgaggagccttcaggattacaagattcaaagtgcgctgctggtgccaaccctattctccttcttcgccaaaagcactctgattgacaaatacgatttatctaatttacacgaaattgcttctggtggcgctcccctctctaaggaagtcggggaagcggttgccaagaggttccatctgccaggtatcaggcaaggatatgggctcactgagactacatcagctattctgattacacccgagggggatgataaaccgggcgcggtcggtaaagttgttccattttttgaagcgaaggttgtggatctggataccgggaaaacgctgggcgttaatcaaagaggcgaactgtgtgtgagaggtcctatgattatgtccggttatgtaaacaatccggaagcgaccaacgccttgattgacaaggatggatggctacattctggagacatagcttactgggacgaagacgaacacttcttcatcgttgaccgcctgaagtctctgattaagtacaaaggctatcaggtggctcccgctgaattggaatccatcttgctccaacaccccaacatcttcgacgcaggtgtcgcaggtcttcccgacgatgacgccggtgaacttcccgccgccgttgttgttttggagcacggaaagacgatgacggaaaaagagatcgtggattacgtcgccagtcaagtaacaaccgcgaaaaagttgcgcggaggagttgtgtttgtggacgaagtaccgaaaggtcttaccggaaaactcgacgcaagaaaaatcagagagatcctcataaaggccaagaagggcggaaagatcgccgtgtaaggtacccgatcagattctagagggccctattctatagtgtcacctaaatgctagagctcgctgatcagcctcgactgtgccttctagttgccagccatctgttgtttgcccctcccccgtgccttccttgaccctggaaggtgccactcccactgtcctttcctaataaaatgaggaaattgcatcgcattgtctgagtaggtgtcattctattctggggggtggggtggggcaggacagcaagggggaggattgggaagacaatagcaggcatgctggggatgcggtgggctctatggcttctgaggcggaaagaaccagctggggctctagggggtatccccacgcgccctgtagcggcgcattaagcgcggcgggtgtggtggttacgcgcagcgtgaccgctacacttgccagcgccctagcgcccgctcctttcgctttcttcccttcctttctcgccacgttcgccggctttccccgtcaagctctaaatcgggggctccctttagggttccgatttagtgctttacggcacctcgaccccaaaaaacttgattagggtgatggttcacgtagtgggccatcgccctgatagacggtttttcgccctttgacgttggagtccacgttctttaatagtggactcttgttccaaactggaacaacactcaaccctatctcggtctattcttttgatttataagggattttgccgatttcggcctattggttaaaaaatgagctgatttaacaaaaatttaacgcgaattaattctgtggaatgtgtgtcagttagggtgtggaaagtccccaggctccccagcaggcagaagtatgcaaagcatgcatctcaattagtcagcaaccaggtgtggaaagtccccaggctccccagcaggcagaagtatgcaaagcatgcatctcaattagtcagcaaccatagtcccgcccctaactccgcccatcccgcccctaactccgcccagttccgcccattctccgccccatggctgactaattttttttatttatgcagaggccgaggccgcctctgcctctgagctattccagaagtagtgaggaggcttttttggaggcctaggcttttgcaaaaagctcccgggagcttgtatatccattttcggatctgatcaagagacaggatgaggatcgtttcgcatgattgaacaagatggattgcacgcaggttctccggccgcttgggtggagaggctattcggctatgactgggcacaacagacaatcggctgctctgatgccgccgtgttccggctgtcagcgcaggggcgcccggttctttttgtcaagaccgacctgtccggtgccctgaatgaactgcaggacgaggcagcgcggctatcgtggctggccacgacgggcgttccttgcgcagctgtgctcgacgttgtcactgaagcgggaagggactggctgctattgggcgaagtgccggggcaggatctcctgtcatctcaccttgctcctgccgagaaagtatccatcatggctgatgcaatgcggcggctgcatacgcttgatccggctacctgcccattcgaccaccaagcgaaacatcgcatcgagcgagcacgtactcggatggaagccggtcttgtcgatcaggatgatctggacgaagagcatcaggggctcgcgccagccgaactgttcgccaggctcaaggcgcgcatgcccgacggcgaggatctcgtcgtgacccatggcgatgcctgcttgccgaatatcatggtggaaaatggccgcttttctggattcatcgactgtggccggctgggtgtggcggaccgctatcaggacatagcgttggctacccgtgatattgctgaagagcttggcggcgaatgggctgaccgcttcctcgtgctttacggtatcgccgctcccgattcgcagcgcatcgccttctatcgccttcttgacgagttcttctgagcgggactctggggttcgaaatgaccgaccaagcgacgcccaacctgccatcacgagatttcgattccaccgccgccttctatgaaaggttgggcttcggaatcgttttccgggacgccggctggatgatcctccagcgcggggatctcatgctggagttcttcgcccaccccaacttgtttattgcagcttataatggttacaaataaagcaatagcatcacaaatttcacaaataaagcatttttttcactgcattctagttgtggtttgtccaaactcatcaatgtatcttatcatgtctgtataccgtcgacctctagctagagcttggcgtaatcatggtcatagctgtttcctgtgtgaaattgttatccgctcacaattccacacaacatacgagccggaagcataaagtgtaaagcctggggtgcctaatgagtgagctaactcacattaattgcgttgcgctcactgcccgctttccagtcgggaaacctgtcgtgccagctgcattaatgaatcggccaacgcgcggggagaggcggtttgcgtattgggcgctcttccgcttcctcgctcactgactcgctgcgctcggtcgttcggctgcggcgagcggtatcagctcactcaaaggcggtaatacggttatccacagaatcaggggataacgcaggaaagaacatgtgagcaaaaggccagcaaaaggccaggaaccgtaaaaaggccgcgttgctggcgtttttccataggctccgcccccctgacgagcatcacaaaaatcgacgctcaagtcagaggtggcgaaacccgacaggactataaagataccaggcgtttccccctggaagctccctcgtgcgctctcctgttccgaccctgccgcttaccggatacctgtccgcctttctcccttcgggaagcgtggcgctttctcatagctcacgctgtaggtatctcagttcggtgtaggtcgttcgctccaagctgggctgtgtgcacgaaccccccgttcagcccgaccgctgcgccttatccggtaactatcgtcttgagtccaacccggtaagacacgacttatcgccactggcagcagccactggtaacaggattagcagagcgaggtatgtaggcggtgctacagagttcttgaagtggtggcctaactacggctacactagaagaacagtatttggtatctgcgctctgctgaagccagttaccttcggaaaaagagttggtagctcttgatccggcaaacaaaccaccgctggtagcggtggtttttttgtttgcaagcagcagattacgcgcagaaaaaaaggatctcaagaagatcctttgatcttttctacggggtctgacgctcagtggaacgaaaactcacgttaagggattttggtcatgagattatcaaaaaggatcttcacctagatccttttaaattaaaaatgaagttttaaatcaatctaaagtatatatgagtaaacttggtctgacagttaccaatgcttaatcagtgaggcacctatctcagcgatctgtctatttcgttcatccatagttgcctgactccccgtcgtgtagataactacgatacgggagggcttaccatctggccccagtgctgcaatgataccgcgagacccacgctcaccggctccagatttatcagcaataaaccagccagccggaagggccgagcgcagaagtggtcctgcaactttatccgcctccatccagtctattaattgttgccgggaagctagagtaagtagttcgccagttaatagtttgcgcaacgttgttgccattgctacaggcatcgtggtgtcacgctcgtcgtttggtatggcttcattcagctccggttcccaacgatcaaggcgagttacatgatcccccatgttgtgcaaaaaagcggttagctccttcggtcctccgatcgttgtcagaagtaagttggccgcagtgttatcactcatggttatggcagcactgcataattctcttactgtcatgccatccgtaagatgcttttctgtgactggtgagtactcaaccaagtcattctgagaatagtgtatgcggcgaccgagttgctcttgcccggcgtcaatacgggataataccgcgccacatagcagaactttaaaagtgctcatcattggaaaacgttcttcggggcgaaaactctcaaggatcttaccgctgttgagatccagttcgatgtaacccactcgtgcacccaactgatcttcagcatcttttactttcaccagcgtttctgggtgagcaaaaacaggaaggcaaaatgccgcaaaaaagggaataagggcgacacggaaatgttgaatactcatactcttcctttttcaatattattgaagcatttatcagggttattgtctcatgagcggatacatatttgaatgtatttagaaaaataaacaaataggggttccgcgcacatttccccgaaaagtgccacctgacgtc

SEQ ID NO: 52 - DNA, 6201 bp, synthetic construct
  source 1..6201: mol_type = other DNA
gacggatcgggagatctcccgatcccctatggtgcactctcagtacaatctgctctgatgccgcatagttaagccagtatctgctccctgcttgtgtgttggaggtcgctgagtagtgcgcgagcaaaatttaagctacaacaaggcaaggcttgaccgacaattgcatgaagaatctgcttagggttaggcgttttgcgctgcttcgcgatgtacgggccagatatacgcgttgacattgattattgactagttattaatagtaatcaattacggggtcattagttcatagcccatatatggagttccgcgttacataacttacggtaaatggcccgcctggctgaccgcccaacgacccccgcccattgacgtcaataatgacgtatgttcccatagtaacgccaatagggactttccattgacgtcaatgggtggagtatttacggtaaactgcccacttggcagtacatcaagtgtatcatatgccaagtacgccccctattgacgtcaatgacggtaaatggcccgcctggcattatgcccagtacatgaccttatgggactttcctacttggcagtacatctacgtattagtcatcgctattaccatggtgatgcggttttggcagtacatcaatgggcgtggatagcggtttgactcacggggatttccaagtctccaccccattgacgtcaatgggagtttgttttggcaccaaaatcaacgggactttccaaaatgtcgtaacaactccgccccattgacgcaaatgggcggtaggcgtgtacggtgggaggtctatataagcagagctctctggctaactagagaacccactgcttactggcttatcgaaattaatacgactcactatagggaaagcttgatcagaacggatccgccaccatggaagacgccaaaaacataaagaaaggcccggcgccattctatccgctggaagatggaaccgctggagagcaactgcataaggctatgaagagatacgccctggttcctggaacaattgcttttacagatgcacatatcgaggtggacatcacttacgctgagtacttcgaaatgtccgttcggttggcagaagctatgaaacgatatgggctgaatacaaatcacagaatcgtcgtatgcagtgaaaactctcttcaattctttatgccggtgttgggcgcgttatttatcggagttgcagttgcgcccgcgaacgacatttataatgaacgtgaattgctcaacagtatgggcatttcgcagcctaccgtggtgttcgtttccaaaaaggggttgcaaaaaattttgaacgtgcaaaaaaagctcccaatcatccaaaaaattattatcatggattctaaaacggattaccagggatttcagtcgatgtacacgttcgtcacatctcatctacctcccggttttaatgaatacgattttgtgccagagtccttcgatagggacaagacaattgcactgatcatgaactcctctggatctactggtctgcctaaaggtgtcgctctgcctcatagaactgcctgcgtgagattctcgcatgccagagatcctatttttggcaatcaaatcattccggatactgcgattttaagtgttgttccattccatcacggttttggaatgtttactacactcggatatttgatatgtggatttcgagtcgtcttaatgtatagatttgaagaagagctgtttctgaggagccttcaggattacaagattcaaagtgcgctgctggtgccaaccctattctccttcttcgccaaaagcactctgattgacaaatacgatttatctaatttacacgaaattgcttctggtggcgctcccctctctaaggaagtcggggaagcggttgccaagaggttccatctgccaggtatcaggcaaggatatgggctcactgagactacatcagctattctgattacacccgagggggatgataaaccgggcgcggtcggtaaagttgttccattttttgaagcgaaggttgtggatctggataccgggaaaacgctgggcgttaatcaaagaggcgaactgtgtgtgagaggtcctatgattatgtccggttatgtaaacaatccggaagcgaccaacgccttgattgacaaggatggatggctacattctggagacatagcttactgggacgaagacgaacacttcttcatcgttgaccgcctgaagtctctgattaagtacaaaggctatcaggtggctcccgctgaattggaatccatcttgctccaacaccccaacatcttcgacgcaggtgtcgcaggtcttcccgacgatgacgccggtgaacttcccgccgccgttgttgttttggagcacggaaagacgatgacggaaaaagagatcgtggattacgtcgccagtcaagtaacaaccgcgaaaaagttgcgcggaggagttgtgtttgtggacgaagtaccgaaaggtcttaccggaaaactcgacgcaagaaaaatcagagagatcctcataaaggccaagaagggcggaaagatcgccgtgtaaggtacccgatcagattctagagggccctattctatagtgtcacctaaatgctagagctcgctgatcagcctcgactgtgccttctagttgccagccatctgttgtttgcccctcccccgtgccttccttgaccctggaaggtgccactcccactgtcctttcctaataaaatgaggaaattgcatcgcattgtctgagtaggtgtcattctattctggggggtggggtggggcaggacagcaagggggaggattgggaagacaatagcaggcatgctggggatgcggtgggctctatggcttctgaggcggaaagaaccagctggggctctagggggtatccccacgcgccctgtagcggcgcattaagcgcggcgggtgtggtggttacgcgcagcgtgaccgctacacttgccagcgccctagcgcccgctcctttcgctttcttcccttcctttctcgccacgttcgccggctttccccgtcaagctctaaatcgggggctccctttagggttccgatttagtgctttacggcacctcgaccccaaaaaacttgattagggtgatggttcacgtagtgggccatcgccctgatagacggtttttcgccctttgacgttggagtccacgttctttaatagtggactcttgttccaaactggaacaacactcaaccctatctcggtctattcttttgatttataagggattttgccgatttcggcctattggttaaaaaatgagctgatttaacaaaaatttaacgcgaattaattctgtggaatgtgtgtcagttagggtgtggaaagtccccaggctccccagcaggcagaagtatgcaaagcatgcatctcaattagtcagcaaccaggtgtggaaagtccccaggctccccagcaggcagaagtatgcaaagcatgcatctcaattagtcagcaaccatagtcccgcccctaactccgcccatcccgcccctaactccgcccagttccgcccattctccgccccatggctgactaattttttttatttatgcagaggccgaggccgcctctgcctctgagctattccagaagtagtgaggaggcttttttggaggcctaggcttttgcaaaaagctcccgggagcttgtatatccattttcggatctgatcaagagacaggatgaggatcgtttcgcgcgggactctggggttcgaaatgaccgaccaagcgacgcccaacctgccatcacgagatttcgattccaccgccgccttctatgaaaggttgggcttcggaatcgttttccgggacgccggctggatgatcctccagcgcggggatctcatgctggagttcttcgcccaccccaacttgtttattgcagcttataatggttacaaataaagcaatagcatcacaaatttcacaaataaagcatttttttcactgcattctagttgtggtttgtccaaactcatcaatgtatcttatcatgtctgtataccgtcgacctctagctagagcttggcgtaatcatggtcatagctgtttcctgtgtgaaattgttatccgctcacaattccacacaacatacgagccggaagcataaagtgtaaagcctggggtgcctaatgagtgagctaactcacattaattgcgttgcgctcactgcccgctttccagtcgggaaacctgtcgtgccagctgcattaatgaatcggccaacgcgcggggagaggcggtttgcgtattgggcgctcttccgcttcctcgctcactgactcgctgcgctcggtcgttcggctgcggcgagcggtatcagctcactcaaaggcggtaatacggttatccacagaatcaggggataacgcaggaaagaacatgtgagcaaaaggccagcaaaaggccaggaaccgtaaaaaggccgcgttgctggcgtttttccataggctccgcccccctgacgagcatcacaaaaatcgacgctcaagtcagaggtggcgaaacccgacaggactataaagataccaggcgtttccccctggaagctccctcgtgcgctctcctgttccgaccctgccgcttaccggatacctgtccgcctttctcccttcgggaagcgtggcgctttctcatagctcacgctgtaggtatctcagttcggtgtaggtcgttcgctccaagctgggctgtgtgcacgaaccccccgttcagcccgaccgctgcgccttatccggtaactatcgtcttgagtccaacccggtaagacacgacttatcgccactggcagcagccactggtaacaggattagcagagcgaggtatgtaggcggtgctacagagttcttgaagtggtggcctaactacggctacactagaagaacagtatttggtatctgcgctctgctgaagccagttaccttcggaaaaagagttggtagctcttgatccggcaaacaaaccaccgctggtagcggtggtttttttgtttgcaagcagcagattacgcgcagaaaaaaaggatctcaagaagatcctttgatcttttctacggggtctgacgctcagtggaacgaaaactcacgttaagggattttggtcatgagattatcaaaaaggatcttcacctagatccttttaaattaaaaatgaagttttaaatcaatctaaagtatatatgagtaaacttggtctgacagttagaaaaactcatcgagcatcaaatgaaactgcaatttattcatatcaggattatcaataccatatttttgaaaaagccgtttctgtaatgaaggagaaaactcaccgaggcagttccataggatggcaagatcctggtatcggtctgcgattccgactcgtccaacatcaatacaacctattaatttcccctcgtcaaaaataaggttatcaagtgagaaatcaccatgagtgacgactgaatccggtgagaatggcaaaagtttatgcatttctttccagacttgttcaacaggccagccattacgctcgtcatcaaaatcactcgcatcaaccaaaccgttattcattcgtgattgcgcctgagcgagacgaaatacgcgatcgctgttaaaaggacaattacaaacaggaatcgaatgcaaccggcgcaggaacactgccagcgcatcaacaatattttcacctgaatcaggatattcttctaatacctggaatgctgttttcccggggatcgcagtggtgagtaaccatgcatcatcaggagtacggataaaatgcttgatggtcggaagaggcataaattccgtcagccagtttagtctgaccatctcatctgtaacatcattggcaacgctacctttgccatgtttcagaaacaactctggcgcatcgggcttcccatacaatcgatagattgtcgcacctgattgcccgacattatcgcgagcccatttatacccatataaatcagcatccatgttggaatttaatcgcggcctagagcaagacgtttcccgttgaatatggctcatactcttcctttttcaatattattgaagcatttatcagggttattgtctcatgagcggatacatatttgaatgtatttagaaaaataaacaaataggggttccgcgcacatttccccgaaaagtgccacctgacgtc

SEQ ID NO: 53 - DNA, 110 bp, synthetic construct
  source 1..110: mol_type = other DNA
aaaaaaaaaaaaaaaaaaaaaaaaaaaaaagcatatgactaaaaaaaaaaaaaaaaaaaaaaaaaaaaaaaaaaaaaaaaaaaaaaaaaaaaaaaaaaaaaaaaaaaaaa

SEQ ID NO: 54 - DNA, 6316 bp, synthetic construct
  source 1..6316: mol_type = other DNA
gacggatcgggagatctcccgatcccctatggtgcactctcagtacaatctgctctgatgccgcatagttaagccagtatctgctccctgcttgtgtgttggaggtcgctgagtagtgcgcgagcaaaatttaagctacaacaaggcaaggcttgaccgacaattgcatgaagaatctgcttagggttaggcgttttgcgctgcttcgcgatgtacgggccagatatacgcgttgacattgattattgactagttattaatagtaatcaattacggggtcattagttcatagcccatatatggagttccgcgttacataacttacggtaaatggcccgcctggctgaccgcccaacgacccccgcccattgacgtcaataatgacgtatgttcccatagtaacgccaatagggactttccattgacgtcaatgggtggagtatttacggtaaactgcccacttggcagtacatcaagtgtatcatatgccaagtacgccccctattgacgtcaatgacggtaaatggcccgcctggcattatgcccagtacatgaccttatgggactttcctacttggcagtacatctacgtattagtcatcgctattaccatggtgatgcggttttggcagtacatcaatgggcgtggatagcggtttgactcacggggatttccaagtctccaccccattgacgtcaatgggagtttgttttggcaccaaaatcaacgggactttccaaaatgtcgtaacaactccgccccattgacgcaaatgggcggtaggcgtgtacggtgggaggtctatataagcagagctctctggctaactagagaacccactgcttactggcttatcgaaattaatacgactcactatagggaaagcttgatcagaacggatccgccaccatggaagacgccaaaaacataaagaaaggcccggcgccattctatccgctggaagatggaaccgctggagagcaactgcataaggctatgaagagatacgccctggttcctggaacaattgcttttacagatgcacatatcgaggtggacatcacttacgctgagtacttcgaaatgtccgttcggttggcagaagctatgaaacgatatgggctgaatacaaatcacagaatcgtcgtatgcagtgaaaactctcttcaattctttatgccggtgttgggcgcgttatttatcggagttgcagttgcgcccgcgaacgacatttataatgaacgtgaattgctcaacagtatgggcatttcgcagcctaccgtggtgttcgtttccaaaaaggggttgcaaaaaattttgaacgtgcaaaaaaagctcccaatcatccaaaaaattattatcatggattctaaaacggattaccagggatttcagtcgatgtacacgttcgtcacatctcatctacctcccggttttaatgaatacgattttgtgccagagtccttcgatagggacaagacaattgcactgatcatgaactcctctggatctactggtctgcctaaaggtgtcgctctgcctcatagaactgcctgcgtgagattctcgcatgccagagatcctatttttggcaatcaaatcattccggatactgcgattttaagtgttgttccattccatcacggttttggaatgtttactacactcggatatttgatatgtggatttcgagtcgtcttaatgtatagatttgaagaagagctgtttctgaggagccttcaggattacaagattcaaagtgcgctgctggtgccaaccctattctccttcttcgccaaaagcactctgattgacaaatacgatttatctaatttacacgaaattgcttctggtggcgctcccctctctaaggaagtcggggaagcggttgccaagaggttccatctgccaggtatcaggcaaggatatgggctcactgagactacatcagctattctgattacacccgagggggatgataaaccgggcgcggtcggtaaagttgttccattttttgaagcgaaggttgtggatctggataccgggaaaacgctgggcgttaatcaaagaggcgaactgtgtgtgagaggtcctatgattatgtccggttatgtaaacaatccggaagcgaccaacgccttgattgacaaggatggatggctacattctggagacatagcttactgggacgaagacgaacacttcttcatcgttgaccgcctgaagtctctgattaagtacaaaggctatcaggtggctcccgctgaattggaatccatcttgctccaacaccccaacatcttcgacgcaggtgtcgcaggtcttcccgacgatgacgccggtgaacttcccgccgccgttgttgttttggagcacggaaagacgatgacggaaaaagagatcgtggattacgtcgccagtcaagtaacaaccgcgaaaaagttgcgcggaggagttgtgtttgtggacgaagtaccgaaaggtcttaccggaaaactcgacgcaagaaaaatcagagagatcctcataaaggccaagaagggcggaaagatcgccgtgtaaggtacccgatcagattctagagggcccaaaaaaaaaaaaaaaaaaaaaaaaaaaaaagcatatgactaaaaaaaaaaaaaaaaaaaaaaaaaaaaaaaaaaaaaaaaaaaaaaaaaaaaaaaaaaaaaaaaaaaaaaagagaccgtctatagtgtcacctaaatgctagagctcgctgatcagcctcgactgtgccttctagttgccagccatctgttgtttgcccctcccccgtgccttccttgaccctggaaggtgccactcccactgtcctttcctaataaaatgaggaaattgcatcgcattgtctgagtaggtgtcattctattctggggggtggggtggggcaggacagcaagggggaggattgggaagacaatagcaggcatgctggggatgcggtgggctctatggcttctgaggcggaaagaaccagctggggctctagggggtatccccacgcgccctgtagcggcgcattaagcgcggcgggtgtggtggttacgcgcagcgtgaccgctacacttgccagcgccctagcgcccgctcctttcgctttcttcccttcctttctcgccacgttcgccggctttccccgtcaagctctaaatcgggggctccctttagggttccgatttagtgctttacggcacctcgaccccaaaaaacttgattagggtgatggttcacgtagtgggccatcgccctgatagacggtttttcgccctttgacgttggagtccacgttctttaatagtggactcttgttccaaactggaacaacactcaaccctatctcggtctattcttttgatttataagggattttgccgatttcggcctattggttaaaaaatgagctgatttaacaaaaatttaacgcgaattaattctgtggaatgtgtgtcagttagggtgtggaaagtccccaggctccccagcaggcagaagtatgcaaagcatgcatctcaattagtcagcaaccaggtgtggaaagtccccaggctccccagcaggcagaagtatgcaaagcatgcatctcaattagtcagcaaccatagtcccgcccctaactccgcccatcccgcccctaactccgcccagttccgcccattctccgccccatggctgactaattttttttatttatgcagaggccgaggccgcctctgcctctgagctattccagaagtagtgaggaggcttttttggaggcctaggcttttgcaaaaagctcccgggagcttgtatatccattttcggatctgatcaagagacaggatgaggatcgtttcgcgcgggactctggggttcgaaatgaccgaccaagcgacgcccaacctgccatcacgagatttcgattccaccgccgccttctatgaaaggttgggcttcggaatcgttttccgggacgccggctggatgatcctccagcgcggggatctcatgctggagttcttcgcccaccccaacttgtttattgcagcttataatggttacaaataaagcaatagcatcacaaatttcacaaataaagcatttttttcactgcattctagttgtggtttgtccaaactcatcaatgtatcttatcatgtctgtataccgtcgacctctagctagagcttggcgtaatcatggtcatagctgtttcctgtgtgaaattgttatccgctcacaattccacacaacatacgagccggaagcataaagtgtaaagcctggggtgcctaatgagtgagctaactcacattaattgcgttgcgctcactgcccgctttccagtcgggaaacctgtcgtgccagctgcattaatgaatcggccaacgcgcggggagaggcggtttgcgtattgggcgctcttccgcttcctcgctcactgactcgctgcgctcggtcgttcggctgcggcgagcggtatcagctcactcaaaggcggtaatacggttatccacagaatcaggggataacgcaggaaagaacatgtgagcaaaaggccagcaaaaggccaggaaccgtaaaaaggccgcgttgctggcgtttttccataggctccgcccccctgacgagcatcacaaaaatcgacgctcaagtcagaggtggcgaaacccgacaggactataaagataccaggcgtttccccctggaagctccctcgtgcgctctcctgttccgaccctgccgcttaccggatacctgtccgcctttctcccttcgggaagcgtggcgctttctcatagctcacgctgtaggtatctcagttcggtgtaggtcgttcgctccaagctgggctgtgtgcacgaaccccccgttcagcccgaccgctgcgccttatccggtaactatcgtcttgagtccaacccggtaagacacgacttatcgccactggcagcagccactggtaacaggattagcagagcgaggtatgtaggcggtgctacagagttcttgaagtggtggcctaactacggctacactagaagaacagtatttggtatctgcgctctgctgaagccagttaccttcggaaaaagagttggtagctcttgatccggcaaacaaaccaccgctggtagcggtggtttttttgtttgcaagcagcagattacgcgcagaaaaaaaggatctcaagaagatcctttgatcttttctacggggtctgacgctcagtggaacgaaaactcacgttaagggattttggtcatgagattatcaaaaaggatcttcacctagatccttttaaattaaaaatgaagttttaaatcaatctaaagtatatatgagtaaacttggtctgacagttagaaaaactcatcgagcatcaaatgaaactgcaatttattcatatcaggattatcaataccatatttttgaaaaagccgtttctgtaatgaaggagaaaactcaccgaggcagttccataggatggcaagatcctggtatcggtctgcgattccgactcgtccaacatcaatacaacctattaatttcccctcgtcaaaaataaggttatcaagtgagaaatcaccatgagtgacgactgaatccggtgagaatggcaaaagtttatgcatttctttccagacttgttcaacaggccagccattacgctcgtcatcaaaatcactcgcatcaaccaaaccgttattcattcgtgattgcgcctgagcgagacgaaatacgcgatcgctgttaaaaggacaattacaaacaggaatcgaatgcaaccggcgcaggaacactgccagcgcatcaacaatattttcacctgaatcaggatattcttctaatacctggaatgctgttttcccggggatcgcagtggtgagtaaccatgcatcatcaggagtacggataaaatgcttgatggtcggaagaggcataaattccgtcagccagtttagtctgaccatctcatctgtaacatcattggcaacgctacctttgccatgtttcagaaacaactctggcgcatcgggcttcccatacaatcgatagattgtcgcacctgattgcccgacattatcgcgagcccatttatacccatataaatcagcatccatgttggaatttaatcgcggcctagagcaagacgtttcccgttgaatatggctcatactcttcctttttcaatattattgaagcatttatcagggttattgtctcatgagcggatacatatttgaatgtatttagaaaaataaacaaataggggttccgcgcacatttccccgaaaagtgccacctgacgtc

SEQ ID NO: 55 - DNA, 170 bp, synthetic construct
  source 1..170: mol_type = other DNA
taatacgactcactataggacagatcgcctggagacgccatccacgctgttttgacctccatagaagacaccgggaccgatccagcctccgcggccgggaacggtgcattggaacgcggattccccgtgccaagagtgacgtaagtaccgcagtcaccgtccttgacacg

SEQ ID NO: 56 - DNA, 74 bp, synthetic construct
  source 1..74: mol_type = other DNA
tcttcacccagtctgtctcttagaatttatttcccactgacacaaacaagccattttgtctgcttgtataaccc